European Patent Application EP 4 428 238 A1, published September 11, 2024. Title: Ligand-binding nucleic acid complex. Applicant: Rena Therapeutics Inc. The sequence listing filed with the application follows.

SEQUENCE LISTING (182 sequences)

SEQ ID NO: 1 - protein, 34 aa, synthetic construct
  REGION 1..34: note = Synthetic
AVSEHQLLHDKGKSIQDLRRRELLEKLLAKLHKA

SEQ ID NO: 2 - protein, 33 aa, synthetic construct
  REGION 1..33: note = Synthetic
VSEHQLLHDKGKSIQDLRRRELLEKLLAKLHKA

SEQ ID NO: 3 - protein, 32 aa, synthetic construct
  REGION 1..32: note = Synthetic
SEHQLLHDKGKSIQDLRRRELLEKLLAKLHKA

SEQ ID NO: 4 - protein, 31 aa, synthetic construct
  REGION 1..31: note = Synthetic
EHQLLHDKGKSIQDLRRRELLEKLLAKLHKA

SEQ ID NO: 5 - protein, 30 aa, synthetic construct
  REGION 1..30: note = Synthetic
HQLLHDKGKSIQDLRRRELLEKLLAKLHKA

SEQ ID NO: 6 - protein, 29 aa, synthetic construct
  REGION 1..29: note = Synthetic
QLLHDKGKSIQDLRRRELLEKLLAKLHKA

SEQ ID NO: 7 - protein, 28 aa, synthetic construct
  REGION 1..28: note = Synthetic
LLHDKGKSIQDLRRRELLEKLLAKLHKA

SEQ ID NO: 8 - protein, 27 aa, synthetic construct
  REGION 1..27: note = Synthetic
LHDKGKSIQDLRRRELLEKLLAKLHKA

SEQ ID NO: 9 - protein, 26 aa, synthetic construct
  REGION 1..26: note = Synthetic
HDKGKSIQDLRRRELLEKLLAKLHKA

SEQ ID NO: 10 - protein, 25 aa, synthetic construct
  REGION 1..25: note = Synthetic
DKGKSIQDLRRRELLEKLLAKLHKA

SEQ ID NO: 11 - protein, 34 aa, synthetic construct
  REGION 1..34: note = Synthetic
AVSEHQLLHDKGKSIQDLRRRELLEKLLAKLHCA

SEQ ID NO: 12 - protein, 33 aa, synthetic construct
  REGION 1..33: note = Synthetic
VSEHQLLHDKGKSIQDLRRRELLEKLLAKLHCA

SEQ ID NO: 13 - protein, 32 aa, synthetic construct
  REGION 1..32: note = Synthetic
SEHQLLHDKGKSIQDLRRRELLEKLLAKLHCA

SEQ ID NO: 14 - protein, 31 aa, synthetic construct
  REGION 1..31: note = Synthetic
EHQLLHDKGKSIQDLRRRELLEKLLAKLHCA

SEQ ID NO: 15 - protein, 30 aa, synthetic construct
  REGION 1..30: note = Synthetic
HQLLHDKGKSIQDLRRRELLEKLLAKLHCA

SEQ ID NO: 16 - protein, 29 aa, synthetic construct
  REGION 1..29: note = Synthetic
QLLHDKGKSIQDLRRRELLEKLLAKLHCA

SEQ ID NO: 17 - protein, 28 aa, synthetic construct
  REGION 1..28: note = Synthetic
LLHDKGKSIQDLRRRELLEKLLAKLHCA

SEQ ID NO: 18 - protein, 27 aa, synthetic construct
  REGION 1..27: note = Synthetic
LHDKGKSIQDLRRRELLEKLLAKLHCA

SEQ ID NO: 19 - protein, 26 aa, synthetic construct
  REGION 1..26: note = Synthetic
HDKGKSIQDLRRRELLEKLLAKLHCA

SEQ ID NO: 20 - protein, 25 aa, synthetic construct
  REGION 1..25: note = Synthetic
DKGKSIQDLRRRELLEKLLAKLHCA

SEQ ID NO: 21 - protein, 34 aa, synthetic construct
  REGION 1..34: note = Synthetic
AVSEHQLLHDKGKSIQDLRRRELLEKLLAKLHTA

SEQ ID NO: 22 - protein, 33 aa, synthetic construct
  REGION 1..33: note = Synthetic
VSEHQLLHDKGKSIQDLRRRELLEKLLAKLHTA

SEQ ID NO: 23 - protein, 32 aa, synthetic construct
  REGION 1..32: note = Synthetic
SEHQLLHDKGKSIQDLRRRELLEKLLAKLHTA

SEQ ID NO: 24 - protein, 31 aa, synthetic construct
  REGION 1..31: note = Synthetic
EHQLLHDKGKSIQDLRRRELLEKLLAKLHTA

SEQ ID NO: 25 - protein, 30 aa, synthetic construct
  REGION 1..30: note = Synthetic
HQLLHDKGKSIQDLRRRELLEKLLAKLHTA

SEQ ID NO: 26 - protein, 29 aa, synthetic construct
  REGION 1..29: note = Synthetic
QLLHDKGKSIQDLRRRELLEKLLAKLHTA

SEQ ID NO: 27 - protein, 28 aa, synthetic construct
  REGION 1..28: note = Synthetic
LLHDKGKSIQDLRRRELLEKLLAKLHTA

SEQ ID NO: 28 - protein, 27 aa, synthetic construct
  REGION 1..27: note = Synthetic
LHDKGKSIQDLRRRELLEKLLAKLHTA

SEQ ID NO: 29 - protein, 26 aa, synthetic construct
  REGION 1..26: note = Synthetic
HDKGKSIQDLRRRELLEKLLAKLHTA

SEQ ID NO: 30 - protein, 25 aa, synthetic construct
  REGION 1..25: note = Synthetic
DKGKSIQDLRRRELLEKLLAKLHTA

SEQ ID NO: 31 - protein, 34 aa, synthetic construct
  REGION 1..34: note = Synthetic
  SITE 29: note = misc_feature - Aib (Aminoisobutyl acid)
AVSEHQLLHDKGKSIQDLRRRELLEKLLXKLHKA

SEQ ID NO: 32 - protein, 33 aa, synthetic construct
  REGION 1..33: note = Synthetic
  SITE 28: note = misc_feature - Aib (Aminoisobutyl acid)
VSEHQLLHDKGKSIQDLRRRELLEKLLXKLHKA

SEQ ID NO: 33 - protein, 32 aa, synthetic construct
  REGION 1..32: note = Synthetic
  SITE 27: note = misc_feature - Aib (Aminoisobutyl acid)
SEHQLLHDKGKSIQDLRRRELLEKLLXKLHKA

SEQ ID NO: 34 - protein, 31 aa, synthetic construct
  REGION 1..31: note = Synthetic
  SITE 26: note = misc_feature - Aib (Aminoisobutyl acid)
EHQLLHDKGKSIQDLRRRELLEKLLXKLHKA

SEQ ID NO: 35 - protein, 30 aa, synthetic construct
  REGION 1..30: note = Synthetic
  SITE 25: note = misc_feature - Aib (Aminoisobutyl acid)
HQLLHDKGKSIQDLRRRELLEKLLXKLHKA

SEQ ID NO: 36 - protein, 29 aa, synthetic construct
  REGION 1..29: note = Synthetic
  SITE 24: note = misc_feature - Aib (Aminoisobutyl acid)
QLLHDKGKSIQDLRRRELLEKLLXKLHKA

SEQ ID NO: 37 - protein, 28 aa, synthetic construct
  REGION 1..28: note = Synthetic
  SITE 23: note = misc_feature - Aib (Aminoisobutyl acid)
LLHDKGKSIQDLRRRELLEKLLXKLHKA

SEQ ID NO: 38 - protein, 27 aa, synthetic construct
  REGION 1..27: note = Synthetic
  SITE 22: note = misc_feature - Aib (Aminoisobutyl acid)
LHDKGKSIQDLRRRELLEKLLXKLHKA

SEQ ID NO: 39 - protein, 26 aa, synthetic construct
  REGION 1..26: note = Synthetic
  SITE 21: note = misc_feature - Aib (Aminoisobutyl acid)
HDKGKSIQDLRRRELLEKLLXKLHKA

SEQ ID NO: 40 - protein, 25 aa, synthetic construct
  REGION 1..25: note = Synthetic
  SITE 20: note = misc_feature - Aib (Aminoisobutyl acid)
DKGKSIQDLRRRELLEKLLXKLHKA

SEQ ID NO: 41 - protein, 34 aa, synthetic construct
  REGION 1..34: note = Synthetic
  SITE 29: note = misc_feature - Aib (Aminoisobutyl acid)
AVSEHQLLHDKGKSIQDLRRRELLEKLLXKLHCA

SEQ ID NO: 42 - protein, 33 aa, synthetic construct
  REGION 1..33: note = Synthetic
  SITE 28: note = misc_feature - Aib (Aminoisobutyl acid)
VSEHQLLHDKGKSIQDLRRRELLEKLLXKLHCA

SEQ ID NO: 43 - protein, 32 aa, synthetic construct
  REGION 1..32: note = Synthetic
  SITE 27: note = misc_feature - Aib (Aminoisobutyl acid)
SEHQLLHDKGKSIQDLRRRELLEKLLXKLHCA

SEQ ID NO: 44 - protein, 31 aa, synthetic construct
  REGION 1..31: note = Synthetic
  SITE 26: note = misc_feature - Aib (Aminoisobutyl acid)
EHQLLHDKGKSIQDLRRRELLEKLLXKLHCA

SEQ ID NO: 45 - protein, 30 aa, synthetic construct
  REGION 1..30: note = Synthetic
  SITE 25: note = misc_feature - Aib (Aminoisobutyl acid)
HQLLHDKGKSIQDLRRRELLEKLLXKLHCA

SEQ ID NO: 46 - protein, 29 aa, synthetic construct
  REGION 1..29: note = Synthetic
  SITE 24: note = misc_feature - Aib (Aminoisobutyl acid)
QLLHDKGKSIQDLRRRELLEKLLXKLHCA

SEQ ID NO: 47 - protein, 28 aa, synthetic construct
  REGION 1..28: note = Synthetic
  SITE 23: note = misc_feature - Aib (Aminoisobutyl acid)
LLHDKGKSIQDLRRRELLEKLLXKLHCA

SEQ ID NO: 48 - protein, 27 aa, synthetic construct
  REGION 1..27: note = Synthetic
  SITE 22: note = misc_feature - Aib (Aminoisobutyl acid)
LHDKGKSIQDLRRRELLEKLLXKLHCA

SEQ ID NO: 49 - protein, 26 aa, synthetic construct
  REGION 1..26: note = Synthetic
  SITE 21: note = misc_feature - Aib (Aminoisobutyl acid)
HDKGKSIQDLRRRELLEKLLXKLHCA

SEQ ID NO: 50 - protein, 25 aa, synthetic construct
  REGION 1..25: note = Synthetic
  SITE 20: note = misc_feature - Aib (Aminoisobutyl acid)
DKGKSIQDLRRRELLEKLLXKLHCA

SEQ ID NO: 51 - protein, 34 aa, synthetic construct
  REGION 1..34: note = Synthetic
  SITE 29: note = misc_feature - Aib (Aminoisobutyl acid)
AVSEHQLLHDKGKSIQDLRRRELLEKLLXKLHTA

SEQ ID NO: 52 - protein, 33 aa, synthetic construct
  REGION 1..33: note = Synthetic
  SITE 28: note = misc_feature - Aib (Aminoisobutyl acid)
VSEHQLLHDKGKSIQDLRRRELLEKLLXKLHTA

SEQ ID NO: 53 - protein, 32 aa, synthetic construct
  REGION 1..32: note = Synthetic
  SITE 27: note = misc_feature - Aib (Aminoisobutyl acid)
SEHQLLHDKGKSIQDLRRRELLEKLLXKLHTA

SEQ ID NO: 54 - protein, 31 aa, synthetic construct
  REGION 1..31: note = Synthetic
  SITE 26: note = misc_feature - Aib (Aminoisobutyl acid)
EHQLLHDKGKSIQDLRRRELLEKLLXKLHTA

SEQ ID NO: 55 - protein, 30 aa, synthetic construct
  REGION 1..30: note = Synthetic
  SITE 25: note = misc_feature - Aib (Aminoisobutyl acid)
HQLLHDKGKSIQDLRRRELLEKLLXKLHTA

SEQ ID NO: 56 - protein, 29 aa, synthetic construct
  REGION 1..29: note = Synthetic
  SITE 24: note = misc_feature - Aib (Aminoisobutyl acid)
QLLHDKGKSIQDLRRRELLEKLLXKLHTA

SEQ ID NO: 57 - protein, 28 aa, synthetic construct
  REGION 1..28: note = Synthetic
  SITE 23: note = misc_feature - Aib (Aminoisobutyl acid)
LLHDKGKSIQDLRRRELLEKLLXKLHTA

SEQ ID NO: 58 - protein, 27 aa, synthetic construct
  REGION 1..27: note = Synthetic
  SITE 22: note = misc_feature - Aib (Aminoisobutyl acid)
LHDKGKSIQDLRRRELLEKLLXKLHTA

SEQ ID NO: 59 - protein, 26 aa, synthetic construct
  REGION 1..26: note = Synthetic
  SITE 21: note = misc_feature - Aib (Aminoisobutyl acid)
HDKGKSIQDLRRRELLEKLLXKLHTA

SEQ ID NO: 60 - protein, 25 aa, synthetic construct
  REGION 1..25: note = Synthetic
  SITE 20: note = misc_feature - Aib (Aminoisobutyl acid)
DKGKSIQDLRRRELLEKLLXKLHTA

SEQ ID NO: 61 - protein, 34 aa, synthetic construct
  REGION 1..34: note = Synthetic
  SITE 29: note = misc_feature - Aib (Aminoisobutyl acid)
  SITE 31: note = misc_feature - Ahc (1-Aminocyclohexylcarboxylic acid)
AVSEHQLLHDKGKSIQDLRRRELLEKLLXKXHTA

SEQ ID NO: 62 - protein, 34 aa, synthetic construct
  REGION 1..34: note = Synthetic
  SITE 23: note = misc_feature - Ahc (1-Aminocyclohexylcarboxylic acid)
  SITE 29: note = misc_feature - Aib (Aminoisobutyl acid)
AVSEHQLLHDKGKSIQDLRRREXLEKLLXKLHTA

SEQ ID NO: 63 - protein, 34 aa, synthetic construct
  REGION 1..34: note = Synthetic
  SITE 27: note = misc_feature - Ahc (1-Aminocyclohexylcarboxylic acid)
  SITE 29: note = misc_feature - Aib (Aminoisobutyl acid)
AVSEHQLLHDKGKSIQDLRRRELLEKXLXKLHTA

SEQ ID NO: 64 - protein, 34 aa, synthetic construct
  REGION 1..34: note = Synthetic
  SITE 30: note = misc_feature - Ahc (1-Aminocyclohexylcarboxylic acid)
AVSEHQLLHDKGKSIQDLRRRELLEKLLEXLHTA

SEQ ID NO: 65 - protein, 34 aa, synthetic construct
  REGION 1..34: note = Synthetic
  SITE 22: note = misc_feature - Cha (2-Amino-3-Cyclohexylpropionic acid)
  SITE 27: note = misc_feature - Ahc (1-Aminocyclohexylcarboxylic acid)
  SITE 29: note = misc_feature - Aib (Aminoisobutyl acid)
AVSEHQLLHDKGKSIQDLRRRXLLEKXLXKLHTA

SEQ ID NO: 66 - protein, 34 aa, synthetic construct
  REGION 1..34: note = Synthetic
  SITE 24: note = misc_feature - Ahc (1-Aminocyclohexylcarboxylic acid)
  SITE 29: note = misc_feature - Aib (Aminoisobutyl acid)
AVSEHQLLHDKGKSIQDLRRRELXEKLLXKLHTA

SEQ ID NO: 67 - protein, 34 aa, synthetic construct
  REGION 1..34: note = Synthetic
  SITE 25: note = misc_feature - Aib (Aminoisobutyl acid)
  SITE 27: note = misc_feature - Ahc (1-Aminocyclohexylcarboxylic acid)
AVSEHQLLHDKGKSIQDLRRRELLXKXLEKLHTA

SEQ ID NO: 68 - protein, 34 aa, synthetic construct
  REGION 1..34: note = Synthetic
  SITE 25: note = misc_feature - Aib (Aminoisobutyl acid)
  SITE 27: note = misc_feature - Ahc (1-Aminocyclohexylcarboxylic acid)
  SITE 29: note = misc_feature - Aib (Aminoisobutyl acid)
AVSEHQLLHDKGKSIQDLRRRELLXKXLXKLHTA

SEQ ID NO: 69 - protein, 34 aa, synthetic construct
  REGION 1..34: note = Synthetic
  SITE 22: note = misc_feature - Ahc (1-Aminocyclohexylcarboxylic acid)
  SITE 29: note = misc_feature - Aib (Aminoisobutyl acid)
AVSEHQLLHDKGKSIQDLRRRXLLEKLLXKLHTA

SEQ ID NO: 70 - protein, 34 aa, synthetic construct
  REGION 1..34: note = Synthetic
  SITE 28: note = misc_feature - Ahc (1-Aminocyclohexylcarboxylic acid)
  SITE 29: note = misc_feature - Aib (Aminoisobutyl acid)
AVSEHQLLHDKGKSIQDLRRRELLEKLXXKLHTA

SEQ ID NO: 71 - protein, 34 aa, synthetic construct
  REGION 1..34: note = Synthetic
  SITE 22: note = misc_feature - Cha (2-Amino-3-Cyclohexylpropionic acid)
  SITE 23: note = misc_feature - Ahc (1-Aminocyclohexylcarboxylic acid)
  SITE 29: note = misc_feature - Aib (Aminoisobutyl acid)
AVSEHQLLHDKGKSIQDLRRRXXLEKLLXKLHTA

SEQ ID NO: 72 - protein, 34 aa, synthetic construct
  REGION 1..34: note = Synthetic
AVSEHQLLHDKGKSIQDLRRRFFLHHLIAEIHTA

SEQ ID NO: 73 - protein, 28 aa, synthetic construct
  REGION 1..28: note = Synthetic
LLHDKGKSIQDLRRRFFLHHLIAEIHTA

SEQ ID NO: 74 - protein, 34 aa, synthetic construct
  REGION 1..34: note = Synthetic
AVSEIQLLHDKGKSIQDLRRRFFLHHLIAEIHTA

SEQ ID NO: 75 - protein, 34 aa, synthetic construct
  REGION 1..34: note = Synthetic
AVSEIQLLHDKGKSIQDLERRFFLHHLIAEIHTA

SEQ ID NO: 76 - protein, 34 aa, synthetic construct
  REGION 1..34: note = Synthetic
AVSEIQLLHDKGKSIQDLRRVFFLHHLIAEIHTA

SEQ ID NO: 77 - protein, 36 aa, synthetic construct
  REGION 1..36: note = Synthetic
AVSEIQLLHDKGKSIQDLRRRFFLHHLIAEIHTAEI

SEQ ID NO: 78 - protein, 36 aa, synthetic construct
  REGION 1..36: note = Synthetic
AVSEHQLLHDKGKSIQDLRRRFFLHHLIAEIHTAEY

SEQ ID NO: 79 - protein, 36 aa, synthetic construct
  REGION 1..36: note = Synthetic
AVSEIQLLHDKGKSIQDLRRRFWLHHLIAEIHTAEY

SEQ ID NO: 80 - protein, 36 aa, synthetic construct
  REGION 1..36: note = Synthetic
AVSEIQLLHDKGKSIQDLRRRFWLHHLIAEIHTAEI

SEQ ID NO: 81 - protein, 35 aa, synthetic construct
  REGION 1..35: note = Synthetic
VSEIQLLHDKGKSIQDLRRRFWLHHLIAEIHTAEI

SEQ ID NO: 82 - protein, 34 aa, synthetic construct
  REGION 1..34: note = Synthetic
SEIQLLHDKGKSIQDLRRRFWLHHLIAEIHTAEI

SEQ ID NO: 83 - protein, 33 aa, synthetic construct
  REGION 1..33: note = Synthetic
EIQLLHDKGKSIQDLRRRFWLHHLIAEIHTAEI

SEQ ID NO: 84 - protein, 32 aa, synthetic construct
  REGION 1..32: note = Synthetic
IQLLHDKGKSIQDLRRRFWLHHLIAEIHTAEI

SEQ ID NO: 85 - protein, 36 aa, synthetic construct
  REGION 1..36: note = Synthetic
AVSEHQLLHDKGKSIQDLRRRFWLHHLIAEIHTAEI

SEQ ID NO: 86 - protein, 36 aa, synthetic construct
  REGION 1..36: note = Synthetic
AVSEHQLLHDKGKSIQDLRRRFWLHHLIAEIHTAEY

SEQ ID NO: 87 - protein, 37 aa, synthetic construct
  REGION 1..37: note = Synthetic
AVSEHQLLHDKGKSIQDLRRRHWLNSYMHKLLVLDAP

SEQ ID NO: 88 - protein, 34 aa, synthetic construct
  REGION 1..34: note = Synthetic
AVSEHQLLHDKGKSIQDLRRREWLRKKLQDVHNF

SEQ ID NO: 89 - protein, 34 aa, synthetic construct
  REGION 1..34: note = Synthetic
SVSEIQLMHNLGKHLNSMERVEWLRKKLQDVHKF

SEQ ID NO: 90 - protein, 33 aa, synthetic construct
  REGION 1..33: note = Synthetic
VSEIQLMHNLGKHLNSMERVEWLRKKLQDVHKF

SEQ ID NO: 91 - protein, 32 aa, synthetic construct
  REGION 1..32: note = Synthetic
SEIQLMHNLGKHLNSMERVEWLRKKLQDVHKF

SEQ ID NO: 92 - protein, 31 aa, synthetic construct
  REGION 1..31: note = Synthetic
EIQLMHNLGKHLNSMERVEWLRKKLQDVHKF

SEQ ID NO: 93 - protein, 30 aa, synthetic construct
  REGION 1..30: note = Synthetic
IQLMHNLGKHLNSMERVEWLRKKLQDVHKF

SEQ ID NO: 94 - protein, 29 aa, synthetic construct
  REGION 1..29: note = Synthetic
QLMHNLGKHLNSMERVEWLRKKLQDVHKF

SEQ ID NO: 95 - protein, 28 aa, synthetic construct
  REGION 1..28: note = Synthetic
LMHNLGKHLNSMERVEWLRKKLQDVHKF

SEQ ID NO: 96 - protein, 27 aa, synthetic construct
  REGION 1..27: note = Synthetic
MHNLGKHLNSMERVEWLRKKLQDVHKF

SEQ ID NO: 97 - protein, 26 aa, synthetic construct
  REGION 1..26: note = Synthetic
HNLGKHLNSMERVEWLRKKLQDVHKF

SEQ ID NO: 98 - protein, 25 aa, synthetic construct
  REGION 1..25: note = Synthetic
NLGKHLNSMERVEWLRKKLQDVHKF

SEQ ID NO: 99 - protein, 34 aa, synthetic construct
  REGION 1..34: note = Synthetic
SVSEIQLMHNLGKHLNSMERVEWLRKKLQDVHCF

SEQ ID NO: 100 - protein, 33 aa, synthetic construct
  REGION 1..33: note = Synthetic
VSEIQLMHNLGKHLNSMERVEWLRKKLQDVHCF

SEQ ID NO: 101 - protein, 32 aa, synthetic construct
  REGION 1..32: note = Synthetic
SEIQLMHNLGKHLNSMERVEWLRKKLQDVHCF

SEQ ID NO: 102 - protein, 31 aa, synthetic construct
  REGION 1..31: note = Synthetic
EIQLMHNLGKHLNSMERVEWLRKKLQDVHCF

SEQ ID NO: 103 - protein, 30 aa, synthetic construct
  REGION 1..30: note = Synthetic
IQLMHNLGKHLNSMERVEWLRKKLQDVHCF

SEQ ID NO: 104 - protein, 29 aa, synthetic construct
  REGION 1..29: note = Synthetic
QLMHNLGKHLNSMERVEWLRKKLQDVHCF

SEQ ID NO: 105 - protein, 28 aa, synthetic construct
  REGION 1..28: note = Synthetic
LMHNLGKHLNSMERVEWLRKKLQDVHCF

SEQ ID NO: 106 - protein, 27 aa, synthetic construct
  REGION 1..27: note = Synthetic
MHNLGKHLNSMERVEWLRKKLQDVHCF

SEQ ID NO: 107 - protein, 26 aa, synthetic construct
  REGION 1..26: note = Synthetic
HNLGKHLNSMERVEWLRKKLQDVHCF

SEQ ID NO: 108 - protein, 25 aa, synthetic construct
  REGION 1..25: note = Synthetic
NLGKHLNSMERVEWLRKKLQDVHCF

SEQ ID NO: 109 - protein, 34 aa, synthetic construct
  REGION 1..34: note = Synthetic
SVSEIQLMHNLGKHLNSMERVEWLRKKLQDVHNF

SEQ ID NO: 110 - protein, 33 aa, synthetic construct
  REGION 1..33: note = Synthetic
VSEIQLMHNLGKHLNSMERVEWLRKKLQDVHNF

SEQ ID NO: 111 - protein, 32 aa, synthetic construct
  REGION 1..32: note = Synthetic
SEIQLMHNLGKHLNSMERVEWLRKKLQDVHNF

SEQ ID NO: 112 - protein, 31 aa, synthetic construct
  REGION 1..31: note = Synthetic
EIQLMHNLGKHLNSMERVEWLRKKLQDVHNF

SEQ ID NO: 113 - protein, 30 aa, synthetic construct
  REGION 1..30: note = Synthetic
IQLMHNLGKHLNSMERVEWLRKKLQDVHNF

SEQ ID NO: 114 - protein, 29 aa, synthetic construct
  REGION 1..29: note = Synthetic
QLMHNLGKHLNSMERVEWLRKKLQDVHNF

SEQ ID NO: 115 - protein, 28 aa, synthetic construct
  REGION 1..28: note = Synthetic
LMHNLGKHLNSMERVEWLRKKLQDVHNF

SEQ ID NO: 116 - protein, 27 aa, synthetic construct
  REGION 1..27: note = Synthetic
MHNLGKHLNSMERVEWLRKKLQDVHNF

SEQ ID NO: 117 - protein, 26 aa, synthetic construct
  REGION 1..26: note = Synthetic
HNLGKHLNSMERVEWLRKKLQDVHNF

SEQ ID NO: 118 - protein, 25 aa, synthetic construct
  REGION 1..25: note = Synthetic
NLGKHLNSMERVEWLRKKLQDVHNF

SEQ ID NO: 119 - protein, 34 aa, synthetic construct
  REGION 1..34: note = Synthetic
  SITE 7: note = misc_feature - Cha (2-Amino-3-Cyclohexylpropionic acid)
  SITE 11: note = misc_feature - Cha (2-Amino-3-Cyclohexylpropionic acid)
SVSEIQXMHNXGKHLNSMERVEWLRKKLQDVHNF

SEQ ID NO: 120 - protein, 34 aa, synthetic construct
  REGION 1..34: note = Synthetic
  SITE 23: note = misc_feature - Cha (2-Amino-3-Cyclohexylpropionic acid)
SVSEIQLMHNLGKHLNSMERVEXLRKKLQDVHNF

SEQ ID NO: 121 - protein, 34 aa, synthetic construct
  REGION 1..34: note = Synthetic
  SITE 24: note = misc_feature - Cha (2-Amino-3-Cyclohexylpropionic acid)
SVSEIQLMHNLGKHLNSMERVEWXRKKLQDVHNF

SEQ ID NO: 122 - protein, 34 aa, synthetic construct
  REGION 1..34: note = Synthetic
  SITE 8: note = misc_feature - Nle (Norleucine)
  SITE 18: note = misc_feature - Nle (Norleucine)
  SITE 27: note = misc_feature - Cha (2-Amino-3-Cyclohexylpropionic acid)
SVSEIQLXHNLGKHLNSXERVEWLRKXLQDVHNF

SEQ ID NO: 123 - protein, 34 aa, synthetic construct
  REGION 1..34: note = Synthetic
  SITE 28: note = misc_feature - Cha (2-Amino-3-Cyclohexylpropionic acid)
SVSEIQLMHNLGKHLNSMERVEWLRKKXQDVHNF

SEQ ID NO: 124 - protein, 34 aa, synthetic construct
  REGION 1..34: note = Synthetic
  SITE 31: note = misc_feature - Cha (2-Amino-3-Cyclohexylpropionic acid)
SVSEIQLMHNLGKHLNSMERVEWLRKKLQDXHNF

SEQ ID NO: 125 - protein, 34 aa, synthetic construct
  REGION 1..34: note = Synthetic
  SITE 16: note = misc_feature - Aib (Aminoisobutyl acid)
SVSEIQLMHNLGKHLXSMERVEWLRKKLQDVHNF

SEQ ID NO: 126 - protein, 34 aa, synthetic construct
  REGION 1..34: note = Synthetic
  SITE 19: note = misc_feature - Aib (Aminoisobutyl acid)
SVSEIQLMHNLGKHLNSMXRVEWLRKKLQDVHNF

SEQ ID NO: 127 - protein, 34 aa, synthetic construct
  REGION 1..34: note = Synthetic
  SITE 34: note = misc_feature - Aib (Aminoisobutyl acid)
SVSEIQLMHNLGKHLNSMERVEWLRKKLQDVHNX

SEQ ID NO: 128 - protein, 34 aa, synthetic construct; identical to SEQ ID NO: 124
  REGION 1..34: note = Synthetic
  SITE 31: note = misc_feature - Nle (Norleucine)

SEQ ID NO: 129 - protein, 34 aa, synthetic construct
  REGION 1..34: note = Synthetic
  SITE 27: note = misc_feature - Homo arginine
SVSEIQLMHNLGKHLNSMERVEWLRKXLQDVHNF

SEQ ID NO: 130 - protein, 34 aa, synthetic construct
  REGION 1..34: note = Synthetic
  SITE 1: note = misc_feature - 2,3-amino propionic acid
  SITE 8: note = misc_feature - Nle (Norleucine)
  SITE 18: note = misc_feature - Nle (Norleucine)
XVSEIQLXHNLGKHLNSXERVEWLRKKLQDVHNY

SEQ ID NO: 131 - protein, 34 aa, synthetic construct
  REGION 1..34: note = Synthetic
  SITE 24: note = misc_feature - Cha (2-Amino-3-Cyclohexylpropionic acid)
  SITE 28: note = misc_feature - Cha (2-Amino-3-Cyclohexylpropionic acid)
  SITE 31: note = misc_feature - Cha (2-Amino-3-Cyclohexylpropionic acid)
SVSEIQLMHNLGKHLNSMERVEWXRKKXQKXHNF

SEQ ID NO: 132 - protein, 34 aa, synthetic construct
  REGION 1..34: note = Synthetic
  SITE 7: note = misc_feature - Cha (2-Amino-3-Cyclohexylpropionic acid)
  SITE 8: note = misc_feature - Nle (Norleucine)
  SITE 11: note = misc_feature - Cha (2-Amino-3-Cyclohexylpropionic acid)
  SITE 18: note = misc_feature - Nle (Norleucine)
SVSEIQXXHNXGKHLNSXERVEWLRKKLQDVHNY

SEQ ID NO: 133 - protein, 34 aa, synthetic construct
  REGION 1..34: note = Synthetic
  SITE 7: note = misc_feature - Cha (2-Amino-3-Cyclohexylpropionic acid)
  SITE 8: note = misc_feature - Nle (Norleucine)
  SITE 11: note = misc_feature - Cha (2-Amino-3-Cyclohexylpropionic acid)
  SITE 16: note = misc_feature - Aib (Aminoisobutyl acid)
  SITE 18: note = misc_feature - Nle (Norleucine)
  SITE 19: note = misc_feature - Aib (Aminoisobutyl acid)
SVSEIQXXHNXGKHLXSXXRVEWLRKKLQDVHNY

SEQ ID NO: 134 - protein, 34 aa, synthetic construct
  REGION 1..34: note = Synthetic
  SITE 7: note = misc_feature - Cha (2-Amino-3-Cyclohexylpropionic acid)
  SITE 8: note = misc_feature - Nle (Norleucine)
  SITE 11: note = misc_feature - Cha (2-Amino-3-Cyclohexylpropionic acid)
  SITE 16: note = misc_feature - Aib (Aminoisobutyl acid)
  SITE 18: note = misc_feature - Nle (Norleucine)
  SITE 19: note = misc_feature - Aib (Aminoisobutyl acid)
  SITE 31: note = misc_feature - Nle (Norleucine)
SVSEIQXXHNXGKHLXSXXRVEWLRKKLQDXHNY

SEQ ID NO: 135 - protein, 34 aa, synthetic construct
  REGION 1..34: note = Synthetic
  SITE 17: note = misc_feature - Cha (2-Amino-3-Cyclohexylpropionic acid)
SVSEIQLMHNLGKHLNXMERVEWLRKKLQDVHNF

SEQ ID NO: 136 - protein, 34 aa, synthetic construct
  REGION 1..34: note = Synthetic
  SITE 28: note = misc_feature - Cha (2-Amino-3-Cyclohexylpropionic acid)
  SITE 31: note = misc_feature - Cha (2-Amino-3-Cyclohexylpropionic acid)
SVSEIQLMHNLGKHLNSMERVEWLRKKXQDXHNF

SEQ ID NO: 137 - protein, 34 aa, synthetic construct
  REGION 1..34: note = Synthetic
  SITE 7: note = misc_feature - Cha (2-Amino-3-Cyclohexylpropionic acid)
  SITE 8: note = misc_feature - Nle (Norleucine)
  SITE 11: note = misc_feature - Cha (2-Amino-3-Cyclohexylpropionic acid)
  SITE 18: note = misc_feature - Nle (Norleucine)
  SITE 34: note = misc_feature - Aib (Aminoisobutyl acid)
SVSEIQXXHNXGKHLNSXERVEWLRKKLQDVHNX

SEQ ID NO: 138 - protein, 34 aa, synthetic construct
  REGION 1..34: note = Synthetic
  SITE 15: note = misc_feature - Cha (2-Amino-3-Cyclohexylpropionic acid)
SVSEIQLMHNLGKHXNSMERVEWLRKKLQDVHNF

SEQ ID NO: 139 - protein, 34 aa, synthetic construct
  REGION 1..34: note = Synthetic
  SITE 7: note = misc_feature - Cha (2-Amino-3-Cyclohexylpropionic acid)
  SITE 11: note = misc_feature - Cha (2-Amino-3-Cyclohexylpropionic acid)
  SITE 19: note = misc_feature - Aib (Aminoisobutyl acid)
SVSEIQXMHNXGKHLNSMXRVEWLRKKLQDVHNF

SEQ ID NO: 140 - protein, 34 aa, synthetic construct
  REGION 1..34: note = Synthetic
  SITE 7: note = misc_feature - Cha (2-Amino-3-Cyclohexylpropionic acid)
  SITE 11: note = misc_feature - Cha (2-Amino-3-Cyclohexylpropionic acid)
  SITE 16: note = misc_feature - Aib (Aminoisobutyl acid)
SVSEIQXMHNXGKHLXSMERVEWLRKKLQDVHNF

SEQ ID NO: 141 - protein, 34 aa, synthetic construct
  REGION 1..34: note = Synthetic
  SITE 16: note = misc_feature - Aib (Aminoisobutyl acid)
  SITE 19: note = misc_feature - Aib (Aminoisobutyl acid)
SVSEIQLMHNLGKHLXSMXRVEWLRKKLQDVHNF

SEQ ID NO: 142 - protein, 34 aa, synthetic construct
  REGION 1..34: note = Synthetic
  SITE 12: note = misc_feature - Aib (Aminoisobutyl acid)
SVSEIQLMHNLXKHLNSMERVEWLRKKLQDVHNF

SEQ ID NO: 143 - protein, 34 aa, synthetic construct
  REGION 1..34: note = Synthetic
  SITE 3: note = misc_feature - Aib (Aminoisobutyl acid)
SVXEIQLMHNLGKHLNSMERVEWLRKKLQDVHNF

SEQ ID NO: 144 - protein, 34 aa, synthetic construct
  REGION 1..34: note = Synthetic
  SITE 7: note = misc_feature - Cha (2-Amino-3-Cyclohexylpropionic acid)
  SITE 11: note = misc_feature - Cha (2-Amino-3-Cyclohexylpropionic acid)
  SITE 19: note = misc_feature - Aib (Aminoisobutyl acid)
SVSEIQXMHNXGKHLNSMXRVEWLRKKLQKVHNF

SEQ ID NO: 145 - protein, 34 aa, synthetic construct
  REGION 1..34: note = Synthetic
  SITE 7: note = misc_feature - Cha (2-Amino-3-Cyclohexylpropionic acid)
SVSEIQXMHNLGKHLNSMERVEWLRKKLQDVHNF

SEQ ID NO: 146 - protein, 34 aa, synthetic construct
  REGION 1..34: note = Synthetic
  SITE 24: note = misc_feature - Cha (2-Amino-3-Cyclohexylpropionic acid)
  SITE 28: note = misc_feature - Cha (2-Amino-3-Cyclohexylpropionic acid)
  SITE 31: note = misc_feature - Cha (2-Amino-3-Cyclohexylpropionic acid)
SVSEIQLMHNLGKHLNSMERVEWXRKKXQDXHNF

SEQ ID NO: 147 - protein, 34 aa, synthetic construct; identical to SEQ ID NO: 135
  REGION 1..34: note = Synthetic
  SITE 17: note = misc_feature - Aib (Aminoisobutyl acid)

SEQ ID NO: 148 - protein, 34 aa, synthetic construct
  REGION 1..34: note = Synthetic
  SITE 7: note = misc_feature - Cha (2-Amino-3-Cyclohexylpropionic acid)
  SITE 11: note = misc_feature - Cha (2-Amino-3-Cyclohexylpropionic acid)
  SITE 15: note = misc_feature - Cha (2-Amino-3-Cyclohexylpropionic acid)
SVSEIQXMHNXGKHXNSMERVEWLRKKLQDVHNF

SEQ ID NO: 149 - protein, 34 aa, synthetic construct
  REGION 1..34: note = Synthetic
SVSEIQLMHNLGKHLNSLERVEWLRKKLQDVHNF

SEQ ID NO: 150 - protein, 34 aa, synthetic construct
  REGION 1..34: note = Synthetic
  SITE 1: note = misc_feature - Aib (Aminoisobutyl acid)
XVSEIQLMHNLGKHLNSMERVEWLRKKLQDVHNF

SEQ ID NO: 151 - protein, 34 aa, synthetic construct
  REGION 1..34: note = Synthetic
SVSEIQLMHNFGKHLNSMERVEWLRKKLQDVHNF

SEQ ID NO: 152 - protein, 34 aa, synthetic construct
  REGION 1..34: note = Synthetic
SVSEIQLLHNLGKHLNSMERVEWLRKKLQDVHNF

SEQ ID NO: 153 - protein, 34 aa, synthetic construct; identical to SEQ ID NO: 142
  REGION 1..34: note = Synthetic
  SITE 12: note = misc_feature - D-Ser

SEQ ID NO: 154 - protein, 34 aa, synthetic construct; identical to SEQ ID NO: 142
  REGION 1..34: note = Synthetic
  SITE 12: note = misc_feature - D-Leu

SEQ ID NO: 155 - protein, 34 aa, synthetic construct
  REGION 1..34: note = Synthetic
  SITE 3: note = misc_feature - Aib (Aminoisobutyl acid)
  SITE 11: note = misc_feature - Homo arginine
AVXEIQLMHQXAKWLNSMRRVEWLRKKLQDVHNF

SEQ ID NO: 156 - protein, 34 aa, synthetic construct
  REGION 1..34: note = Synthetic
SVSEIQLMHNLGKHLNSMRRVEWLRKKLQDVHNF

SEQ ID NO: 157 - protein, 34 aa, synthetic construct
  REGION 1..34: note = Synthetic
SVSEIQLMHNLGKHLNSMERVEWLRKKLQDVHNY

SEQ ID NO: 158 - protein, 32 aa, synthetic construct
  REGION 1..32: note = Synthetic
SEIQLMHNLGKHLNSMERVEWLRKKLQDVHNY

SEQ ID NO: 159 - protein, 34 aa, synthetic construct
  REGION 1..34: note = Synthetic
SVSEIQLMHNLGKHLNSMERVEFLRKKLQDVHNF

SEQ ID NO: 160 - protein, 34 aa, synthetic construct
  REGION 1..34: note = Synthetic
  SITE 8: note = misc_feature - Nle (Norleucine)
  SITE 18: note = misc_feature - Nle (Norleucine)
AVSEIQFXHNLGKHLSSXERVEWLRKKLQDVHNY

SEQ ID NO: 161 - protein, 32 aa, synthetic construct
  REGION 1..32: note = Synthetic
  SITE 6: note = misc_feature - Nle (Norleucine)
  SITE 16: note = misc_feature - Nle (Norleucine)
SEIQFXHNLGKHLSSXERVEWLRKKLQDVHNY

SEQ ID NO: 162 - protein, 28 aa, synthetic construct
  REGION 1..28: note = Synthetic
  SITE 6: note = misc_feature - D-Trp
FMHNLXKHLSSMERVEWLRKKLQDVHNY

SEQ ID NO: 163 - protein, 34 aa, synthetic construct
  REGION 1..34: note = Synthetic
AVSEIQLMHNLGKHLASVERMQWLRKKLQDVHNF

SEQ ID NO: 164 - protein, 34 aa, synthetic construct
  REGION 1..34: note = Synthetic
  SITE 8: note = misc_feature - Nle (Norleucine)
  SITE 21: note = misc_feature - Nle (Norleucine)
AVSEIQLXHNLGKHLASVERXQWLRKKLQDVHNY

SEQ ID NO: 165 - protein, 39 aa, synthetic construct
  REGION 1..39: note = Synthetic
SLALADDAAFRERARLLAALERRHWLNSYMHKLLVLDAP

SEQ ID NO: 166 - protein, 37 aa, synthetic construct
  REGION 1..37: note = Synthetic
ALADDAAFRERARLLAALERRHWLNSYMHKLLVLDAP

SEQ ID NO: 167 - protein, 33 aa, synthetic construct
  REGION 1..33: note = Synthetic
DAAFRERARLLAALERRHWLNSYMHKLLVLDAP

SEQ ID NO: 168 - protein, 31 aa, synthetic construct
  REGION 1..31: note = Synthetic
AFRERARLLAALERRHWLNSYMHKLLVLDAP

SEQ ID NO: 169 - DNA, 14 bp, synthetic construct
  misc_feature 1..14: note = Synthetic
  source 1..14: mol_type = other DNA
aatgcacgtgggcc

SEQ ID NO: 170 - RNA, 14 nt, synthetic construct
  misc_feature 1..14: note = Synthetic
  source 1..14: mol_type = other RNA
ggcccacgtgcatt

SEQ ID NO: 171 - DNA, 13 bp, synthetic construct
  misc_feature 1..13: note = Synthetic
  source 1..13: mol_type = other DNA
gcattggtattca

SEQ ID NO: 172 - RNA, 13 nt, synthetic construct
  misc_feature 1..13: note = Synthetic
  source 1..13: mol_type = other RNA
tgaataccaatgc

SEQ ID NO: 173 - DNA, 16 bp, synthetic construct
  misc_feature 1..16: note = Synthetic
  source 1..16: mol_type = other DNA
acaataaataccgagg

SEQ ID NO: 174 - RNA, 16 nt, synthetic construct
  misc_feature 1..16: note = Synthetic
  source 1..16: mol_type = other RNA
cctcggtatttattgt

SEQ ID NO: 175 - DNA, 25 bp, synthetic construct
  misc_feature 1..25: note = Synthetic
  source 1..25: mol_type = other DNA
ggccaaacctcggcttacctgaaat

SEQ ID NO: 176 - RNA, 26 nt, synthetic construct
  misc_feature 1..26: note = Synthetic
  source 1..26: mol_type = other RNA
atttcaggtaagccgaggtttaggcc

SEQ ID NO: 177 - RNA, 20 nt, synthetic construct
  misc_feature 1..20: note = Synthetic
  source 1..20: mol_type = other RNA
gcacacttccaatacttacc

SEQ ID NO: 178 - RNA, 20 nt, synthetic construct
  misc_feature 1..20: note = Synthetic
  source 1..20: mol_type = other RNA
ggtaagtattggaagtgtgc

SEQ ID NO: 179 - DNA, 16 bp, synthetic construct
  misc_feature 1..16: note = Synthetic
  source 1..16: mol_type = other DNA
ctagttcactgaatgc

SEQ ID NO: 180 - RNA, 16 nt, synthetic construct
  misc_feature 1..16: note = Synthetic
  source 1..16: mol_type = other RNA
gcattcagtgaactag

SEQ ID NO: 181 - RNA, 23 nt, synthetic construct
  misc_feature 1..23: note = Synthetic
  source 1..23: mol_type = other RNA
attgtcattgagagcaatgccag

SEQ ID NO: 182 - RNA, 21 nt, synthetic construct
  misc_feature 1..21: note = Synthetic
  source 1..21: mol_type = other RNA
ggcattgctctcaatgacaat